European Patent Application EP 4 299 731 A1, published January 3, 2024. Title: Synthetic DNA primase-polymerase and uses thereof. Applicant: ASOCIACIÓN CENTRO DE INVESTIGACIÓN COOPERATIVA EN NANOCIENCIAS "CIC nanoGUNE". The sequence listing filed with the application follows.

SEQUENCE LISTING (6 sequences)

SEQ ID NO: 1 - protein, 298 aa, Artificial
  Artificial DNA primase-polymerase
RAPHSSPLEAALGYARLGYPVLPLLPGEKRPHPRLVPHGLKEASQDPATLEAWWRSCPEAGVGILAPAGVLVLDFDDPTAWEGLRQEHPALEAAPRQRTPKGGVHVFLRLPEGVRLSASVRAIPGVDLRGMGRAYVVAAPTRLKDGRTYSWEVPLVRPAELPPVPEALLARLLPPPPPPPREVWTPVEGASPKRLRALLEAYAHRVAATPPGTRHNTLIRYAVAAGGLIPHGLDPREAEEALVAAALSAGLPEREARAAVRWGLEVGRSRPLDLESSLPPRLPWTYRGRVYARVRRWA

SEQ ID NO: 2 - protein, 298 aa, Artificial
  Artificial DNA primase-polymerase
AHSTSPLEAALGYARMGYPVLPVAPGSKRPHPRLVPHGLKEASTDPATIEAWWRSCPEANVGILAPEGVLVLDLDDPTAWEGLRQLHPALLAAPRARTPRGGVHLYLRLPPGVRLSASVRALPGVDLRGMGRAYVVAAPSRLKDGRTYAWVVPLRRPSELPPVPQALLARLLAPPPPPAARPVSTPVEGASPKRLRALLEAACHRVAHTPPGQRHNTLIRHAVAVGGLIPHGLDQEEAEEALVAAALSAGLPEREARAAVRWGLEAGASRPLVLKPSLPPRLRWTIRRRVRARGRRHG

SEQ ID NO: 3 - protein, 298 aa, Artificial
  Artificial DNA primase-polymerase
ALSTSPLEAALGYARMGYPVLPVAPGSKRPHPRLVRHGLKEATTDPALIEAWWSSRPEANVGILPPAGVLVLDLDSPAGWAGLRQLHPALLAAPRARTPGGGVHLYFRLPPGVRLSASVRVLPGVDLRGMGRAYVVAPPSRHADGRTYEWVVPLRRPSELPPVPQALLALLLAPPPPPAARPVSTPVASARPKAYRAALEAECDRVARTPPGQRHNTLIRHAVALGGLIPRGLDQEEVEGALLAAALRAGLPEREARAAIRWGLEAGASRPLALKPRLPPRLRWTIRRRARARGRRHG

SEQ ID NO: 4 - protein, 298 aa, Artificial
  Artificial DNA primase-polymerase
ALSTSPLEAALAYARMGYPVLPVAPGSKRPHPRLVRHGLKEATTDPAQIEAWWSRRPEANVGILTPSGVLVLDLDSPDGWAGLRQLHPALLPAPKVRTPGGGVHLYFRLPPGVRLRASVRVLPGIDLRGMGRAYVVAPPSRHAHGRTYEWVVPLRAPSELPPVPQALLALLLAPPPPPAARPVSPPVASARPDAYRAALEAECDRVARTPPGQRHNTLIRHAVALGGLVPRGLDEEEVEGALLAAALRAGLAEREARATIRWGLEAGASRPLDLRPRLPPRLRWRIRRRARARGRRHG

SEQ ID NO: 5 - DNA, 20 bp, Artificial
  Primer
cagctcactcaaaggcggta

SEQ ID NO: 6 - DNA, 20 bp, Artificial
  Primer
tctgctctgatgccgcatag